European Patent Application EP 4 613 777 A1, published September 10, 2025. Title: IMMUNE-CELL-TARGETING ANTIBODY OR FUNCTIONAL FRAGMENT THEREOF, AND APPLICATION THEREOF. Applicant: GUANGDONG KEYANGLE LIFE TECHNOLOGY CO., LTD. Application EP. The sequence listing filed with the application follows.

SEQUENCE LISTING (31 sequences)

SEQ ID NO: 1 - protein, 23 aa, Gallus gallus
LQPDPGAVAAAAVLRAVLEGLQG

SEQ ID NO: 2 - protein, 26 aa, Rattus norvegicus
DQPDPGAVAAAAIFRAILEVLQTKAA

SEQ ID NO: 3 - protein, 26 aa, Canis lupus
DQPDPGAVAAAAILRTILEVLQSQGV

SEQ ID NO: 4 - protein, 26 aa, Sus scrofa
DQPDPGAVAAAAILRAILEVLQSQGA

SEQ ID NO: 5 - protein, 26 aa, Bos taurus
DQPDPGAVAAAAILRAILEVLQSQGA

SEQ ID NO: 6 - protein, 23 aa, Macaca mulatta
EQPDPGAVAAAAILRAILEVLQS

SEQ ID NO: 7 - protein, 27 aa, Mus musculus
LDQPDPGAVAAAAIFRAILEVLQTQGA

SEQ ID NO: 8 - protein, 8 aa, Homo sapiens
AILEVLQS

SEQ ID NO: 9 - protein, 10 aa, Homo sapiens
LRAILEVLQS

SEQ ID NO: 10 - protein, 11 aa, Homo sapiens
ILRAILEVLQS

SEQ ID NO: 11 - protein, 13 aa, Homo sapiens
AAILRAILEVLQS

SEQ ID NO: 12 - protein, 23 aa, Homo sapiens
EQPDPGAVAAAAILRAILEVLQS

SEQ ID NO: 13 - protein, 19 aa, Homo sapiens
PGAVAAAAILRAILEVLQS

SEQ ID NO: 14 - protein, 41 aa, Homo sapiens
KNMEAGAGRASYISSARLEQPDPGAVAAAAILRAILEVLQS

SEQ ID NO: 15 - protein, 8 aa, synthetic construct
AVLEVLQG

SEQ ID NO: 16 - protein, 11 aa, synthetic construct
VLRAVLEVLQG

SEQ ID NO: 17 - protein, 23 aa, synthetic construct
EQPDPSAVAAAAILRAILEVLQG

SEQ ID NO: 18 - protein, 23 aa, synthetic construct
LQPDPSAVAAAAVLRAVLEVLQG

SEQ ID NO: 19 - protein, 445 aa, synthetic construct
DVKIVESGGGLVKLGGSLKLSCAASGFTFSRNYMSWVRQTPEKRLELVAGINNNGGSTYYPDTVKGRFTISRDNAKNTLYLQMSSLRSEDTAIYYCAKRGFITTVGAMDYWGQGISVTVSSAKTTPPSVYPLAPGSAAQTNSMVTLGCLVKGYFPEPVTVTWNSGSLSSGVHTFPAVLQSDLYTLSSSVTVPSSTWPSETVTCNVAHPASSTKVDKKIVPRDCGCKPCICTVPEVSSVFIFPPKPKDVLTITLTPKVTCVVVDISKDDPEVQFSWFVDDVEVHTAQTQPREEQFNSTFRSVSELPIMHQDWLNGKEFKCRVNSAAFPAPIEKTISKTKGRPKAPQVYTIPPPKEQMAKDKVSLTCMITDFFPEDITVEWQWNGQPAENYKNTQPIMDTDGSYFVYSKLNVQKSNWEAGNTFTCSVLHEGLHNHHTEKSLSHSPGK

SEQ ID NO: 20 - DNA, 1338 bp, synthetic construct
  source 1..1338: mol_type = other DNA
gatgtgaagatagtggaaagtggtggtggattggtcaaacttggggggtccctgaaactcagctgcgctgccagcggcttcacatttagtagaaactacatgtcctgggtgaggcaaacgccagagaagcggctggagcttgtagctggcatcaacaacaatggaggcagcacctactatcctgacacagtcaaaggacgcttcaccatatccagagacaatgcaaagaataccctgtatctgcagatgtcatctttacgatcagaagatactgcaatctattactgtgccaagaggggttttattacaactgtgggggccatggactactggggccagggcatttctgttactgtgtcctccgccaagaccacaccaccttccgtctatcccttggcaccaggatcagccgcccaaactaacagtatggtgacactgggatgcctggttaagggctatttccctgagccagtgacagtgacttggaacagtggtagcctgagttcaggggtccacactttccccgctgtcttgcagagtgatctgtataccctcagctcctcagtgaccgttcctagcagtacgtggccttccgagactgtgacatgtaatgtagcccatcccgcttcatctaccaaggtggataagaagattgttccacgggactgcgggtgtaaaccgtgtatttgtactgtacccgaggtgagttccgttttcattttccctcccaagcccaaagatgttctcacaattactctgacaccaaaagttacatgcgtggtggtggacatcagcaaggacgatcctgaggtgcagttttcctggtttgttgatgacgtcgaagtccacactgcacagacccagccaagggaagaacagttcaatagtacattcagatccgtgtccgaattgccgattatgcatcaggactggctcaatggcaaagaatttaagtgtagagtgaactctgccgcctttcctgctcctatcgaaaagacaatcagcaagactaagggcagacctaaagccccccaagtgtatactattccaccccccaaagaacagatggccaaggacaaagtaagtttgacctgtatgatcactgacttcttcccagaagatatcactgtggaatggcagtggaacggacagcctgcggagaactataaaaatactcagcccattatggacacagacgggtcttacttcgtctacagtaaactgaatgttcagaaaagtaattgggaggccggcaatacattcacctgttcagtgctgcatgaggggcttcacaaccaccacactgagaaatcccttagccacagccctggcaagtaa

SEQ ID NO: 21 - protein, 214 aa, synthetic construct
DIQMTQTTFSLSASLGDRVTISCRASQDISNYLNWYQQIPDGTVKLLIYYTSRLHSGVPSRFSGSGSGTDYSLTISNLEQEDIATYFCQQVHTLPYTFGGGTKLEMKRADAAPTVSIFPPSSEQLTSGGASVVCFLNNFYPKDINVKWKIDGSERQNGVLNSWTDQDSKDSTYSMSSTLTLTKDEYERHNSYTCEATHKTSTSPIVKSFNRNEC

SEQ ID NO: 22 - DNA, 645 bp, synthetic construct
  source 1..645: mol_type = other DNA
gacattcagatgacccagacgaccttcagcctctctgcatcccttggagacagagtcaccatcagctgtcgggccagccaagatatatcaaattatctgaactggtaccagcagatcccagatggcactgtgaagctgcttatctactacacatcacgcctacattctggtgttccttccaggttttctgggagtggcagtgggacagactattccctcaccattagcaacctggagcaggaagatattgctacttacttctgccagcaagtgcacacactgccctatacttttggaggtggcaccaaattggagatgaaacgggccgatgctgctcctaccgtcagtatcttcccaccttcaagcgaacagcttaccagtggcggggcatctgtggtgtgcttcctgaataacttttacccaaaggatataaacgtgaagtggaagatcgacggcagcgagcggcaaaatggagtgttgaatagttggactgaccaggactctaaggactccacctactctatgtcatctacacttacactgacaaaggatgagtacgaacggcacaactcctatacatgcgaagctacccataagaccagtaccagccccattgtgaagtcattcaatagaaatgagtgctaa

SEQ ID NO: 23 - DNA, 52 bp, synthetic construct
  source 1..52: mol_type = other DNA
ggcctccggactctagaggatccgccaccatggagacagacacactcctgct

SEQ ID NO: 24 - DNA, 39 bp, synthetic construct
  source 1..39: mol_type = other DNA
ctcgagctaagcttcgaattcttacttgccagggctgtg

SEQ ID NO: 25 - DNA, 57 bp, synthetic construct
  source 1..57: mol_type = other DNA
cagaattcgaagcttagctcgagagccaccatggagacagacacactcctgctatgg

SEQ ID NO: 26 - DNA, 42 bp, synthetic construct
  source 1..42: mol_type = other DNA
cagaggttgattgtcgagatatcaaactcattactaaccggt

SEQ ID NO: 27 - protein, 19 aa, synthetic construct
KEQPDPGAVAAAAILRAIL

SEQ ID NO: 28 - protein, 22 aa, synthetic construct
KEQPDPGAVAAAAILRAILEVL

SEQ ID NO: 29 - protein, 24 aa, synthetic construct
KEQPDPGAVAAAAILRAILEVLQS

SEQ ID NO: 30 - protein, 23 aa, synthetic construct
EQPDPGAVAAAAILRAILEVLQS

SEQ ID NO: 31 - protein, 28 aa, synthetic construct
SSARLEQPDPGAVAAAAILRAILEVLQS